European Patent Application EP 4 455 280 A1, published October 30, 2024. Title: Mutated lysophospholipase and mutated Aspergillus niger strain for expressing the enzyme. Applicant: WILMAR (SHANGHAI) BIOTECHNOLOGY RESEARCH & DEVELOPMENT CENTER CO., LTD. The sequence listing filed with the application follows.

SEQUENCE LISTING (21 sequences)

SEQ ID NO: 1 - DNA, 20 bp, synthetic construct
  source 1..20: mol_type = other DNA
atgtttctccgcagggaatt

SEQ ID NO: 2 - DNA, 20 bp, synthetic construct
  source 1..20: mol_type = other DNA
ctacgagcattcactaatgt

SEQ ID NO: 3 - DNA, 1072 bp, Aspergillus niger
  source 1..1072: mol_type = genomic DNA
atgtttctccgcagggaatttggggctgttgcagccctatctgtgctggcccatgctgctcccgcacctgctccgatgcagcgtagaggtaagacacacttaccaatttgcagaacacccgctaacctactcagacatctcctctaccgtcttggacaatatcgacctcttcgcccaatacagtgcagcagcttactgctcctcgaacatcgagtccaccggcacgactctgacctgcgacgtaggcaattgccctctcgtcgaggcagccggtgccacgaccatcgatgagtttgacgagtaagccaatccaaccccaacatcttcccccacttggcatccagctcacacccccatagcaccagcagctacggcgacccgactgggttcatcgccgttgacccaacgaacgagttaattgttctgtctttccggggtagttccgacctctcgaactggattgccgacctagacttcggcctcacctccgtaagcagcatctgtgatggctgtgagatgcacaagggcttctacgaggcctgggaagtcatcgcggacaccatcactagcaaggtggaggctgctgtctccagctatccggactacaccctcgtgttcactggacacagctacggcgctgcattggcggctgtcgcggccaccgtgctccgcaacgccggatacactcttgacctggtaagttcctactcttttatccttgtaacgttcccccatcattcggatggtctactaacacaatcaacagtacaacttcggccagccccgtattggcaacctcgccttagccgactatatcaccggccaaaatatgggcagcaactaccgcgtcacgcacaccgatgacatcgtgcctaagctgcctccggagctgctgggctaccaccacttcagcccggagtactggatcaccagcggtaatgatgtgacggtgactacgtcggacgtgaccgaggtcgtgggggtggattcgacggctgggaatgacggcacgctgcttgacagtacgactgcccatcggtggtacacgatctacattagtgaatgctcgtag

SEQ ID NO: 4 - protein, 298 aa, Aspergillus niger
MFLRREFGAVAALSVLAHAAPAPAPMQRRDISSTVLDNIDLFAQYSAAAYCSSNIESTGTTLTCDVGNCPLVEAAGATTIDEFDDTSSYGDPTGFIAVDPTNELIVLSFRGSSDLSNWIADLDFGLTSVSSICDGCEMHKGFYEAWEVIADTITSKVEAAVSSYPDYTLVFTGHSYGAALAAVAATVLRNAGYTLDLYNFGQPRIGNLALADYITGQNMGSNYRVTHTDDIVPKLPPELLGYHHFSPEYWITSGNDVTVTTSDVTEVVGVDSTAGNDGTLLDSTTAHRWYTIYISECS

SEQ ID NO: 5 - protein, 279 aa, synthetic construct
APAPAPMQRRDISSTVLDNIDLFAQYSAAAYCSSNIESTGTTLTCDVGNCPLVEAAGATTIDEFDDTSSYGDPTGFIAVDPTNELIVLSFRGSSDLSNWIADLDFGLTSVSSICDGCEMHKGFYEAWEVIADTITSKVEAAVSSYPDYTLVFTGHSYGAALAAVAATVLRNAGYTLDLYNFGQPRIGNLALADYITGQNMGSNYRVTHTDDIVPKLPPELLGYHHFSPEYWITSGNDVTVTTSDVTEVVGVDSTAGNDGTLLDSTTAHRWYTIYISECS

SEQ ID NO: 6 - DNA, 840 bp, synthetic construct
  source 1..840: mol_type = other DNA
gctccagctcctgcaccaatgcaaagaagagatatttcttctaccgttttggataacattgatttgttcgctcaatactccgctgctgcttactgttcttctaacattgagtctactggtaccactttgacttgtgacgttggtaactgtccattggttgaggctgctggtgctaccactattgatgagttcgatgatacttcctcttacggtgatcctactggtttcattgctgttgaccctactaacgagttgattgttttgtcttttagaggttcttctgacttgtctaactggattgctgatttggatttcggtttgacttctgtttcttctatttgtgacggttgtgaaatgcacaagggtttctatgaagcctgggaagttattgctgatactattacttctaaggttgaagctgctgtttcttcttacccagattacactttggttttcaccggtcactcttacggtgctgccttggctgctgttgctgctactgttttgagaaacgctggttacactttggatttgtacaactttggtcaaccaagaattggtaacttggctttggctgactacattactggtcaaaacatgggttctaactacagagttactcacactgatgatattgttcctaagttgccaccagagttgttgggttaccaccacttctccccagagtactggattacttctggtaacgatgttactgttaccacttctgatgttactgaggttgttggtgttgattccaccgctggtaacgatggtactttgttggactctactactgctcacagatggtacaccatttacatttctgagtgttcttaa

SEQ ID NO: 7 - DNA, 30 bp, synthetic construct
  source 1..30: mol_type = other DNA
tccccgcggcgaaacgatgagatttccttc

SEQ ID NO: 8 - DNA, 28 bp, synthetic construct
  source 1..28: mol_type = other DNA
ccggaattcttaagaacactcagaaatg

SEQ ID NO: 9 - DNA, 21 bp, synthetic construct
  source 1..21: mol_type = other DNA
gactggttccaattgacaagc

SEQ ID NO: 10 - DNA, 24 bp, synthetic construct
  source 1..24: mol_type = other DNA
ggcaaatggcattctgacatcctc

SEQ ID NO: 11 - protein, 279 aa, synthetic construct
APAPAPMQRRDISSTVLDNIDLFAQYSAAAYCSSNIESTGTTLTCDVGNCPLVEAAGATTIDEFDDTSSYGDPTGFIAVDPTNELIVLSFRGSSDISNWIADLDFGLTSVSSICDGCEMHKGFYEAWEVIADTITSKVEAAVSSYPDYTLVFTGHSYGAALAAVAATVLRNAGYTLDLYNFGQPRIGNLALADYITDQNMGSNYRVTHTDDIVPKLPPKLLGYHHFSPEYWITSGNDVTVTTSDVTEVVGVDSTDGNDGTLLDSTTAHRWYTIYISECS

SEQ ID NO: 12 - DNA, 840 bp, synthetic construct
  source 1..840: mol_type = other DNA
gctccagctcctgcaccaatgcaaagaagagatatttcttctaccgttttggataacattgatttgttcgctcaatactccgctgctgcttactgttcttctaacattgagtctactggtaccactttgacttgtgacgttggtaactgtccattggttgaggctgctggtgctaccactattgatgagttcgatgatacttcctcttacggtgatcctactggtttcattgctgttgaccctactaacgagttgattgttttgtcttttagaggttcttctgacatctctaactggattgctgatttggatttcggtttgacttctgtttcttctatttgtgacggttgtgaaatgcacaagggtttctatgaagcctgggaagttattgctgatactattacttctaaggttgaagctgctgtttcttcttacccagattacactttggttttcaccggtcactcttacggtgctgccttggctgctgttgctgctactgttttgagaaacgctggttacactttggatttgtacaactttggtcaaccaagaattggtaacttggctttggctgactacattactgatcaaaacatgggttctaactacagagttactcacactgatgatattgttcctaagttgccaccaaagttgttgggttaccaccacttctccccagagtactggattacttctggtaacgatgttactgttaccacttctgatgttactgaggttgttggtgttgattccaccgatggtaacgatggtactttgttggactctactactgctcacagatggtacaccatttacatttctgagtgttcttaa

SEQ ID NO: 13 - protein, 279 aa, synthetic construct
APAPAPMQRRDISSTVLDNIDLFAQYSAAAYCSSNIESTGTTLTCDVGNCPLVEAAGATTIDEFDDTSSYGDPTGFIAVDPTNELIVLSFRGSSDISNWIADLDFGLTSVSSICDGCEMHKGFYEAWEVIADTITSKVEAAVSSYPDYTLVFTGHSYGAALAAVAATVLRNAGYTLDLYNFGQPRIGNLALADYITDQNMGSNYRVTHTDDIVPKLPPKLLGYHHFSPEYWITSGNDVTVTTSDVTEVVGVDSTDGNDGTLLDSWTAHRWYTIYISECS

SEQ ID NO: 14 - protein, 269 aa, synthetic construct
DISSTVLDNIDLFAQYSAAAYCSSNIESTGTTLTCDVGNCPLVEAAGATTIDEFDDTSSYGDPTGFIAVDPTNELIVLSFRGSSDISNWIADLDFGLTSVSSICDGCEMHKGFYEAWEVIADTITSKVEAAVSSYPDYTLVFTGHSYGAALAAVAATVLRNAGYTLDLYNFGQPRIGNLALADYITDQNMGSNYRVTHTDDIVPKLPPKLLGYHHFSPEYWITSGNDVTVTTSDVTEVVGVDSTDGNDGTLLDSWTAHRWYTIYISECS

SEQ ID NO: 15 - protein, 279 aa, synthetic construct
APAPAPMQRRDISSTVLDNIDLFAQYSAAAYCSSNIESTGTTLTCDVGNCPLVEAAGATTIDEFDDTSSYGDPTGFIAVDPTNELIVLSFRGSSDISNWIADLDFGLTSVSSICDGCEMHKGFYEAWEVIADTITSKVEAAVSSYPDYTLVFTGHSYGAALAAVAATVLRNAGYTLDLYNFGQPRIGNLALADYITDQNMGSNYRVTHTDDIVPKLPPKLLGYHHFSPEYWITSGNDVTVTTSDVTEVVGVDSTDGNDGTLLDSFTAHRWYTIYISECS

SEQ ID NO: 16 - protein, 269 aa, synthetic construct
DISSTVLDNIDLFAQYSAAAYCSSNIESTGTTLTCDVGNCPLVEAAGATTIDEFDDTSSYGDPTGFIAVDPTNELIVLSFRGSSDISNWIADLDFGLTSVSSICDGCEMHKGFYEAWEVIADTITSKVEAAVSSYPDYTLVFTGHSYGAALAAVAATVLRNAGYTLDLYNFGQPRIGNLALADYITDQNMGSNYRVTHTDDIVPKLPPKLLGYHHFSPEYWITSGNDVTVTTSDVTEVVGVDSTDGNDGTLLDSFTAHRWYTIYISECS

SEQ ID NO: 17 - protein, 279 aa, synthetic construct
APAPAPMQRRDISSTVLDNIDLFAQYSAAAYCSSNIESTGTTLTCDVGNCPLVEAAGATTIDEFDDTSSYGDPTGFIAVDPTNELIVLSFRGSSDISNWIADLDFGLTSVSSICDGCEMHKGFYEAWEVIADTITSKVEAAVSSYPDYTLVFTGHSYGAALAAVAATVLRNAGYTLDLYNFGQPRIGNLALADYITDQNMGSNYRVTHTDDIVPKLPPKLLGYHHFSPEYWITSGNDVTVTTSDVTEVVGVDSTDGNDGTLLDSYTAHRWYTIYISECS

SEQ ID NO: 18 - protein, 269 aa, synthetic construct
DISSTVLDNIDLFAQYSAAAYCSSNIESTGTTLTCDVGNCPLVEAAGATTIDEFDDTSSYGDPTGFIAVDPTNELIVLSFRGSSDISNWIADLDFGLTSVSSICDGCEMHKGFYEAWEVIADTITSKVEAAVSSYPDYTLVFTGHSYGAALAAVAATVLRNAGYTLDLYNFGQPRIGNLALADYITDQNMGSNYRVTHTDDIVPKLPPKLLGYHHFSPEYWITSGNDVTVTTSDVTEVVGVDSTDGNDGTLLDSYTAHRWYTIYISECS

SEQ ID NO: 19 - DNA, 1015 bp, Aspergillus niger
  source 1..1015: mol_type = genomic DNA
gctcccgcacctgctccgatgcagcgtagaggtaagacacacttaccaatttgcagaacacccgctaacctactcagacatctcctctaccgtcttggacaatatcgacctcttcgcccaatacagtgcagcagcttactgctcctcgaacatcgagtccaccggcacgactctgacctgcgacgtaggcaattgccctctcgtcgaggcagccggtgccacgaccatcgatgagtttgacgagtaagccaatccaaccccaacatcttcccccacttggcatccagctcacacccccatagcaccagcagctacggcgacccgactgggttcatcgccgttgacccaacgaacgagttaattgttctgtctttccggggtagttccgacctctcgaactggattgccgacctagacttcggcctcacctccgtaagcagcatctgtgatggctgtgagatgcacaagggcttctacgaggcctgggaagtcatcgcggacaccatcactagcaaggtggaggctgctgtctccagctatccggactacaccctcgtgttcactggacacagctacggcgctgcattggcggctgtcgcggccaccgtgctccgcaacgccggatacactcttgacctggtaagttcctactcttttatccttgtaacgttcccccatcattcggatggtctactaacacaatcaacagtacaacttcggccagccccgtattggcaacctcgccttagccgactatatcaccggccaaaatatgggcagcaactaccgcgtcacgcacaccgatgacatcgtgcctaagctgcctccggagctgctgggctaccaccacttcagcccggagtactggatcaccagcggtaatgatgtgacggtgactacgtcggacgtgaccgaggtcgtgggggtggattcgacggctgggaatgacggcacgctgcttgacagtacgactgcccatcggtggtacacgatctacattagtgaatgctcgtag

SEQ ID NO: 20 - protein, 279 aa, Aspergillus niger; identical to SEQ ID NO: 5

SEQ ID NO: 21 - DNA, 43 bp, synthetic construct
  source 1..43: mol_type = other DNA
gtcgtgtcgggcatttatcgggggatggaccaatcagcgtagg